European Patent Specification EP 3 097 114 B1, published April 10, 2024. Title: Interaction of Draxin and gamma-Netrins. Applicant: Max-Planck-Gesellschaft zur Förderung der Wissenschaften e.V. The sequence listing filed with the application follows.

SEQUENCE LISTING (81 sequences)

SEQ ID NO: 1 - protein, 21 aa, Homo sapiens
EVMPTLDMALFDWTDYEDLKP

SEQ ID NO: 2 - protein, 21 aa, Danio rerio
DVAPTFNMALFDWTDYEDMRP

SEQ ID NO: 3 - protein, 21 aa, Danio rerio
EVMPTLDMTLFDWTDYEDMKP

SEQ ID NO: 4 - protein, 349 aa, Homo sapiens
MAGPAIHTAPMLFLVLLLPLELSLAGALAPGTPARNLPENHIDLPGPALWTPQASHHRRRGPGKKEWGPGLPSQAQDGAVVTATRQASRLPEAEGLLPEQSPAGLLQDKDLLLGLALPYPEKENRPPGWERTRKRSREHKRRRDRLRLHQGRALVRGPSSLMKKAELSEAQVLDAAMEESSTSLAPTMFFLTTFEAAPATEESLILPVTSLRPQQAQPRSDGEVMPTLDMALFDWTDYEDLKPDGWPSAKKKEKHRGKLSSDGNETSPAEGEPCDHHQDCLPGTCCDLREHLCTPHNRGLNNKCFDDCMCVEGLRCYAKFHRNRRVTRRKGRCVEPETANGDQGSFINV

SEQ ID NO: 5 - protein, 360 aa, Danio rerio
MVAPGLCQLFILLLITLSHTLHSSEISSDNFKQSLTPSTTTSKEHPETGLTGGRQQKRHWSGKERDSAGLFSQRHMDRLEDDGTSMEGLSPVRLEMGPGDTMKAEVHGEVRASAQMRQGSHPAEGELNRKGRRHSHRLLAEHRKHGGKKDKGRGKGDLSDPEPELDSLLKDLNAFEDGLNTSPPNYNSVPLNEVPSPLSPILVTTAIKGHPPTLPPASTKPQKSSQGRTQGEVMPTLDMTLFDWTDYEDMKPADSWPSNKRKDKRRSKNKSNGNTTTEAGIVEPCDHHLDCLSGSCCDLREFECKPHNRGLNNKCFDDCMCEEGLRCYAKFHRKRRVTRRRGRCVDPESVNSNQGAFITV

SEQ ID NO: 6 - protein, 351 aa, Danio rerio
MAVSCWYFALFLIFDLMTMTLGTNTHHNSPMEVFSENIIIPPKPEASIHHHTHQRTDRGRKERMTASQLRERPRIAIFHTQNEGPDLEGLSPVRLEMEPADKRRVMTPRKKTFMGSDSLIQEKMNISPGAETPEKAMRRPTVRKVFGGHITRAPHEEESLASGKKRRVSFDQRLNKASFGSPTEPVLPAATVGTFILPITAAVDGNPNPSSEPQVRRYLGGDVAPTFNMALFDWTDYEDMRPGDKKQYSKKQGSEKQATQSPSTGLVRLTSENNVCKHHLDCLPGSCCNLRKHVCELHNRGFNNKCYDSCMCEEGLRCYAKSHRHYRITRKKGQCVDPEDLNHAVSRWMQM

SEQ ID NO: 7 - protein, 75 aa, Danio rerio
HPPTLPPASTKPQKSSQGRTQGEVMPTLDMTLFDWTDYEDMKPADSWPSNKRKDKRRSKNKSNGNTTTEAGIVEP

SEQ ID NO: 8 - protein, 66 aa, Danio rerio
HPPTLPPASTKPQKSSQGRTQGEVMPTLDMTLFDWTDYEDMKPADSWPSNKRKDKRRSKNKSNGNT

SEQ ID NO: 9 - protein, 48 aa, Danio rerio
HPPTLPPASTKPQKSSQGRTQGEVMPTLDMTLFDWTDYEDMKPADSWP

SEQ ID NO: 10 - protein, 43 aa, Danio rerio
HPPTLPPASTKPQKSSQGRTQGEVMPTLDMTLFDWTDYEDMKP

SEQ ID NO: 11 - protein, 50 aa, Danio rerio
QGRTQGEVMPTLDMTLFDWTDYEDMKPADSWPSNKRKDKRRSKNKSNGNT

SEQ ID NO: 12 - protein, 32 aa, Danio rerio
QGRTQGEVMPTLDMTLFDWTDYEDMKPADSWP

SEQ ID NO: 13 - protein, 27 aa, Danio rerio
QGRTQGEVMPTLDMTLFDWTDYEDMKP

SEQ ID NO: 14 - protein, 22 aa, Danio rerio
GEVMPTLDMTLFDWTDYEDMKP

SEQ ID NO: 15 - protein, 21 aa, Danio rerio
EVMPTLDMTLFDWTDYEDMKP

SEQ ID NO: 16 - protein, 22 aa, Homo sapiens
GEVMPTLDMALFDWTDYEDLKP

SEQ ID NO: 17 - protein, 22 aa, Danio rerio
GDVAPTFNMALFDWTDYEDMRP

SEQ ID NO: 18 - DNA, 1047 bp, Homo sapiens
atggctgggcctgccatccacaccgctcccatgctgttcctcgtcctcctgctgcccctggagctgagcctggcaggcgcccttgcacctgggacccctgcccggaacctccctgagaatcacattgacctcccaggcccagcgctgtggacgcctcaggccagccaccaccgccggcggggcccgggcaagaaggagtggggcccaggcctgcccagccaggcccaggatggggctgtggtcaccgccaccaggcaggcctccaggctgccagaggctgaggggctgctgcctgagcagagtcctgcaggcctgctgcaggacaaggacctgctcctgggactggcattgccctaccccgagaaggagaaccgacctccaggttgggagaggaccaggaaacgcagcagggagcacaagagacgcagggacaggttgaggctgcaccaaggccgagccttggtccgaggtcccagctccctgatgaagaaggcagagctctccgaagcccaggtgctggatgcagccatggaggaatcctccaccagcctggcgcccaccatgttctttctcaccacctttgaggcagcacctgccacagaagagtccctgatcctgcccgtcacctccctgcggccccagcaggcacagcccaggtctgacggggaggtgatgcccacgctggacatggccttgttcgactggaccgattatgaagacttaaaacctgatggttggccctctgcaaagaagaaagagaaacaccgcggtaaactctccagtgatggtaacgaaacatcaccagccgaaggggaaccatgcgaccatcaccaagactgcctgccagggacttgctgcgacctgcgggagcatctctgcacaccccacaaccgaggcctcaacaacaaatgcttcgatgactgcatgtgtgtggaagggctgcgctgctatgccaaattccaccggaaccgcagggttacacggaggaaagggcgctgtgtggagcccgagacggccaacggcgaccagggatccttcatcaacgtc

SEQ ID NO: 19 - DNA, 1080 bp, Danio rerio
atggtggctcctggcttgtgtcaactcttcattctacttcttataacactgtctcacactttgcacagctctgaaatctcatctgacaatttcaaacagagtctgaccccctccaccactacctccaaggaacaccctgaaacaggacttaccggtggcagacaacaaaagagacactggtcaggcaaagaacgggatagtgctgggctgttttctcaaaggcatatggacagactggaggatgatgggacaagtatggagggtctgagccccgtaaggctagagatgggacctggggacactatgaaggcagaagttcacggtgaggtcagggcttctgctcaaatgcgtcaaggaagtcatccagcagaaggagagttaaatcgtaaaggcagacgacatagtcacaggcttctggctgagcacagaaagcatggaggcaaaaaagacaaaggtcgaggtaaaggggatctcagcgaccctgaaccagaattagactccttgctgaaggacttaaatgcatttgaggatggtctaaacacttctccacccaattacaacagtgtccctctcaatgaagttccctcccctctctcccctattttggtaaccacggcaatcaaagggcatcccccaacacttcccccagcctccaccaaaccccagaagtcaagccaaggcaggactcaaggtgaagtgatgcccactctggacatgaccctctttgactggactgattatgaggatatgaagcctgcagacagttggccatcaaacaaaagaaaagataaacgtcgcagcaaaaacaagagcaatggaaacacaacaactgaggctggaattgttgaaccatgtgaccatcatcttgactgcctttctggttcctgttgtgacctcagagaatttgaatgtaaacctcacaaccgtggcctaaataacaagtgttttgatgactgcatgtgtgaggagggtctccgatgttacgccaagttccaccgcaagcggagagtgacccgaagacgtggccgctgtgtggaccctgaatcagtcaacagcaaccaaggagcttttattaccgtc

SEQ ID NO: 20 - DNA, 1053 bp, Danio rerio
atggcagtttcctgttggtattttgccttatttctcatctttgacttgatgactatgacactgggcaccaacacccaccacaattcaccaatggaagtcttcagcgaaaacataataatcccgcccaagccagaggcatccatacatcatcacactcatcaaaggacagacagaggacgcaaggagaggatgacagccagtcagctcagagaaagaccccgcattgccatcttccacacccaaaatgaagggccagacctggagggcctcagtcccgttcgcttagagatggaaccggcagacaaacgtcgggtaatgactcctagaaagaagaccttcatgggctctgattccttaattcaagaaaaaatgaatatttctcctggtgccgagactccagagaaggcgatgaggcgtcccactgttcgaaaagtgtttggagggcacatcactagggctcctcatgaggaagagtctttggcatcagggaagaaacggagggtttcttttgatcaaaggctcaataaagcctcctttgggagtcccacagagccagtgcttcctgctgccactgttggcaccttcatattgcccataactgcagcagtcgatgggaatccaaacccctcaagtgaaccgcaggtcagacgttatttaggtggggatgtggcgcccacttttaacatggccttatttgactggacggattatgaagatatgaggcctggagataaaaagcaatattcgaaaaagcaaggttctgaaaaacaggctacacaaagcccaagcactggacttgtgagacttacatcagaaaacaatgtctgtaaacatcatctggattgtctgccaggttcctgctgcaatctcagaaagcatgtgtgtgagcttcataaccgtggcttcaataacaagtgctatgacagctgcatgtgtgaggaaggacttcggtgctatgcaaaatcacacagacattaccgcatcacccgcaaaaagggacagtgtgttgatcctgaggacctaaatcatgcagtcagcagatggatgcagatg

SEQ ID NO: 21 - DNA, 303 bp, Danio rerio
atggtggctcctggcttgtgtcaactcttcattctacttcttataacactgtctcacactttgcacagctctgaagggcatcccccaacacttcccccagcctccaccaaaccccagaagtcaagccaaggcaggactcaaggtgaagtgatgcccactctggacatgaccctctttgactggactgattatgaggatatgaagcctgcagacagttggccatcaaacaaaagaaaagataaacgtcgcagcaaaaacaagagcaatggaaacacaacaactgaggctggaattgttgaacca

SEQ ID NO: 22 - protein, 101 aa, Danio rerio
MVAPGLCQLFILLLITLSHTLHSSEGHPPTLPPASTKPQKSSQGRTQGEVMPTLDMTLFDWTDYEDMKPADSWPSNKRKDKRRSKNKSNGNTTTEAGIVEP

SEQ ID NO: 23 - DNA, 276 bp, Danio rerio
atggtggctcctggcttgtgtcaactcttcattctacttcttataacactgtctcacactttgcacagctctgaagggcatcccccaacacttcccccagcctccaccaaaccccagaagtcaagccaaggcaggactcaaggtgaagtgatgcccactctggacatgaccctctttgactggactgattatgaggatatgaagcctgcagacagttggccatcaaacaaaagaaaagataaacgtcgcagcaaaaacaagagcaatggaaacaca

SEQ ID NO: 24 - protein, 92 aa, Danio rerio
MVAPGLCQLFILLLITLSHTLHSSEGHPPTLPPASTKPQKSSQGRTQGEVMPTLDMTLFDWTDYEDMKPADSWPSNKRKDKRRSKNKSNGNT

SEQ ID NO: 25 - DNA, 222 bp, Danio rerio
atggtggctcctggcttgtgtcaactcttcattctacttcttataacactgtctcacactttgcacagctctgaagggcatcccccaacacttcccccagcctccaccaaaccccagaagtcaagccaaggcaggactcaaggtgaagtgatgcccactctggacatgaccctctttgactggactgattatgaggatatgaagcctgcagacagttggcca

SEQ ID NO: 26 - protein, 74 aa, Danio rerio
MVAPGLCQLFILLLITLSHTLHSSEGHPPTLPPASTKPQKSSQGRTQGEVMPTLDMTLFDWTDYEDMKPADSWP

SEQ ID NO: 27 - DNA, 207 bp, Danio rerio
atggtggctcctggcttgtgtcaactcttcattctacttcttataacactgtctcacactttgcacagctctgaagggcatcccccaacacttcccccagcctccaccaaaccccagaagtcaagccaaggcaggactcaaggtgaagtgatgcccactctggacatgaccctctttgactggactgattatgaggatatgaagcct

SEQ ID NO: 28 - protein, 69 aa, Danio rerio
MVAPGLCQLFILLLITLSHTLHSSEGHPPTLPPASTKPQKSSQGRTQGEVMPTLDMTLFDWTDYEDMKP

SEQ ID NO: 29 - DNA, 225 bp, Danio rerio
atggtggctcctggcttgtgtcaactcttcattctacttcttataacactgtctcacactttgcacagctctgaacaaggcaggactcaaggtgaagtgatgcccactctggacatgaccctctttgactggactgattatgaggatatgaagcctgcagacagttggccatcaaacaaaagaaaagataaacgtcgcagcaaaaacaagagcaatggaaacaca

SEQ ID NO: 30 - protein, 75 aa, Danio rerio
MVAPGLCQLFILLLITLSHTLHSSEQGRTQGEVMPTLDMTLFDWTDYEDMKPADSWPSNKRKDKRRSKNKSNGNT

SEQ ID NO: 31 - DNA, 171 bp, Danio rerio
atggtggctcctggcttgtgtcaactcttcattctacttcttataacactgtctcacactttgcacagctctgaacaaggcaggactcaaggtgaagtgatgcccactctggacatgaccctctttgactggactgattatgaggatatgaagcctgcagacagttggcca

SEQ ID NO: 32 - protein, 57 aa, Danio rerio
MVAPGLCQLFILLLITLSHTLHSSEQGRTQGEVMPTLDMTLFDWTDYEDMKPADSWP

SEQ ID NO: 33 - DNA, 156 bp, Danio rerio
atggtggctcctggcttgtgtcaactcttcattctacttcttataacactgtctcacactttgcacagctctgaacaaggcaggactcaaggtgaagtgatgcccactctggacatgaccctctttgactggactgattatgaggatatgaagcct

SEQ ID NO: 34 - protein, 52 aa, Danio rerio
MVAPGLCQLFILLLITLSHTLHSSEQGRTQGEVMPTLDMTLFDWTDYEDMKP

SEQ ID NO: 35 - DNA, 141 bp, Danio rerio
atggtggctcctggcttgtgtcaactcttcattctacttcttataacactgtctcacactttgcacagctctgaaggtgaagtgatgcccactctggacatgaccctctttgactggactgattatgaggatatgaagcct

SEQ ID NO: 36 - protein, 47 aa, Danio rerio
MVAPGLCQLFILLLITLSHTLHSSEGEVMPTLDMTLFDWTDYEDMKP

SEQ ID NO: 37 - DNA, 1809 bp, Danio rerio
atggtgagagtctctgatgctttggtcactttggtgactctctgctgtgtgctcaaagggactgtcggcggatatggaatgagcatgttcgccgctcagacctccccgccggatccgtgttacgacgagaacggacaccccagaagatgcatccccgacttcgtaaacgcggcgttcgggaaagaagtacgcgcgtccagcacctgcggcaaaacgccgagtcgttactgcgtggtgaccgagaaaggggacgaaagacacagaaactgccacacgtgcgacgcgtcagacccaaagaagaatcacccaccagcttacctgaccgacctgaacaatcctcacaatctcacctgctggcagtcggacaattacctccagtatcctcaaaacgtcactttaactttatccttgggcaagaaatttgaggtgacctacgtgagtttgcagttctgctcacctcgaccggagtctatggcgatctttaaatcgatggactacggaaagtcctgggtgcctttccagtactactcgacccagtgtagaaagatgtacaacaagcccagcaaagccacgattactaagcagaacgagcaagaggccatctgcacagattctcacaccgacatgcatcctctctccggcgggctgatcgcgttcagcaccctggacgggcgaccctccgcgcacgactttgacaattcacccgtacttcaggactgggtgaccgccactgacattaaggtgactttcagccgcctgcacactttcggagacgaaaacgaggatgactcggagctggccagagattcctatttttacgcagtttccgacctgcaggttggaggcagatgtaagtgtaatggacacgcatcacggtgcgtcaaagaccgggatggaaacctagtgtgcgagtgcaagcacaacacagccggaccagagtgtgacagatgcaaaccttttcactatgaccgaccctggcagcgcgcaaccgccagagaagccaacgaatgtgtcgcctgcaattgtaaccttcatgcgaggcgctgtcgtttcaacatggagctttacaaactctctggaaggaaaagtggaggagtctgtctgaactgccgccacaatacagctggtcgccactgccactactgcaaagagggctactatagagacatgtccaagcccatctcccacagaaaggcctgcaaagcctgtgattgccatcctgtgggggccgcgggcaaaacctgtaaccaaaccacaggccaatgcccctgtaaagacggtgtgacgggtatcacatgcaaccgttgtgctaacggctaccagcagagccgatcacccattgccccctgcataaaaattcccatcgctccgccaaccaccactgcaagcagcacagaagagccatcagactgtgaatcctactgcaaggcatccaaaggcaagctgaagatcaatatgaagaagtactgcaagaaagattatgccgttcaagtccacatcctgaaagcagataaagcaggagagtggtggaagttcaccgtcaacatcatctctgtttacaaacagggtgaaagccgaattcgcagaggagaccagttcctctgggtcagggcaaaggatgtggcctgcaagtgtccgaagatcaagtccggcaagaaataccttctgctggggaacgacgaggattcgccaggacaaagcggaatggtggcggacaagggcagtctggtcattcagtggagagacacttgggctcggagactccggaagtttcagcaaagggagaagaaaggaaaatgcaagaaagca

SEQ ID NO: 38 - protein, 603 aa, Danio rerio
MVRVSDALVTLVTLCCVLKGTVGGYGMSMFAAQTSPPDPCYDENGHPRRCIPDFVNAAFGKEVRASSTCGKTPSRYCVVTEKGDERHRNCHTCDASDPKKNHPPAYLTDLNNPHNLTCWQSDNYLQYPQNVTLTLSLGKKFEVTYVSLQFCSPRPESMAIFKSMDYGKSWVPFQYYSTQCRKMYNKPSKATITKQNEQEAICTDSHTDMHPLSGGLIAFSTLDGRPSAHDFDNSPVLQDWVTATDIKVTFSRLHTFGDENEDDSELARDSYFYAVSDLQVGGRCKCNGHASRCVKDRDGNLVCECKHNTAGPECDRCKPFHYDRPWQRATAREANECVACNCNLHARRCRFNMELYKLSGRKSGGVCLNCRHNTAGRHCHYCKEGYYRDMSKPISHRKACKACDCHPVGAAGKTCNQTTGQCPCKDGVTGITCNRCANGYQQSRSPIAPCIKIPIAPPTTTASSTEEPSDCESYCKASKGKLKINMKKYCKKDYAVQVHILKADKAGEWWKFTVNIISVYKQGESRIRRGDQFLWVRAKDVACKCPKIKSGKKYLLLGNDEDSPGQSGMVADKGSLVIQWRDTWARRLRKFQQREKKGKCKKA

SEQ ID NO: 39 - DNA, 1374 bp, Danio rerio
atggtaaggattttggtaacgtgcgtctccatggtgtccatcacctcgatggtgtccggtgctcgcggtggatacgggatgagcatgttcgcggctcagtcctctcctccggacccgtgctacgacgagaacgggaaccccagacgctgcatccccgacttcgtgaactccgctttcgggaaggacgtgcgcgtgtccagcacctgcggctctcctccgtcgcgctactgcgtggtgaccgagaaaggcgaggagagatcgagggactgcaacatctgcgacgccacagaccccaaaaagacccatccgcccgcatacctgacagacctcaacaaccctcataacctcacctgctggcagtcggagaactacgtgcaatacccgcagaacgtgactctgactctgtctttggggaagaagtttgaagtgacttatgtgagcctccagttctgctctcctcgccccgaatccatggccatcttcaaatccatggactatgggaaaacctgggtgccttttcagttctactcaacccagtgcaagaaaatgtacaacaagcccagcaaagctgccatcaccaagcagaacgagcaggaggcgatctgcacggactctcacacggacatgcagccgttaaccggcggcctcatcgcgttcagcacgctggatggcagaccgtccgcgcacgacttcgacaactcgcccgtcctgcaggactgggtcacggccaccgacatcaaagtgaccttcaaccggctgcacacgttcggggatgagaacgaggacgattcggagctcgccagggactcgtatttttacgcggtgtctgacctgcaggtcggtggacggtgtaagtgtaacgggcacgcgtcgaagtgcgtgaaggaccgggaaggaaacctagtgtgcgaatgcaagcacaacactgcgggaccagagtgtgacaggtgtaaacccttccactacgaccggccctggcagcgcgcgactgccagagaggcgaacgagtgtgtcgcttgtcactgtaacctacatgcccgccgctgccgcttcaacatggagctgtataagttgtcaggccgcaggagtggaggagtctgcctgaactgcagacacaacaccgccggacgccactgccactactgtaaagagggctactacagagacatgagcaaggctatatcacaccgacgtgcatgcaaagcctgcgattgtcatcctgttggtgcagctggtaagacctgtaaccagacaactggacagtgtccatgtaaagatggtgtgactggcatcacctgtaatcgctgtgctaaaggataccagcagagcagatcacccatcgccccctgtatcaaaattccagttgctgctccc

SEQ ID NO: 40 - protein, 458 aa, Danio rerio
MVRILVTCVSMVSITSMVSGARGGYGMSMFAAQSSPPDPCYDENGNPRRCIPDFVNSAFGKDVRVSSTCGSPPSRYCVVTEKGEERSRDCNICDATDPKKTHPPAYLTDLNNPHNLTCWQSENYVQYPQNVTLTLSLGKKFEVTYVSLQFCSPRPESMAIFKSMDYGKTWVPFQFYSTQCKKMYNKPSKAAITKQNEQEAICTDSHTDMQPLTGGLIAFSTLDGRPSAHDFDNSPVLQDWVTATDIKVTFNRLHTFGDENEDDSELARDSYFYAVSDLQVGGRCKCNGHASKCVKDREGNLVCECKHNTAGPECDRCKPFHYDRPWQRATAREANECVACHCNLHARRCRFNMELYKLSGRRSGGVCLNCRHNTAGRHCHYCKEGYYRDMSKAISHRRACKACDCHPVGAAGKTCNQTTGQCPCKDGVTGITCNRCAKGYQQSRSPIAPCIKIPVAAP

SEQ ID NO: 41 - DNA, 1374 bp, Danio rerio
atggtgagagtctctgatgctttggtcactttggtgactctctgctgtgtgctcaaagggactgtcggcggatatggaatgagcatgttcgccgctcagacctccccgccggatccgtgttacgacgagaacggacaccccagaagatgcatccccgacttcgtaaacgcggcgttcgggaaagaagtacgcgcgtccagcacctgcggcaaaacgccgagtcgttactgcgtggtgaccgagaaaggggacgaaagacacagaaactgccacacgtgcgacgcgtcagacccaaagaagaatcacccaccagcttacctgaccgacctgaacaatcctcacaatctcacctgctggcagtcggacaattacctccagtatcctcaaaacgtcactttaactttatccttgggcaagaaatttgaggtgacctacgtgagtttgcagttctgctcacctcgaccggagtctatggcgatctttaaatcgatggactacggaaagtcctgggtgcctttccagtactactcgacccagtgtagaaagatgtacaacaagcccagcaaagccacgattactaagcagaacgagcaagaggccatctgcacagattctcacaccgacatgcatcctctctccggcgggctgatcgcgttcagcaccctggacgggcgaccctccgcgcacgactttgacaattcacccgtacttcaggactgggtgaccgccactgacattaaggtgactttcagccgcctgcacactttcggagacgaaaacgaggatgactcggagctggccagagattcctatttttacgcagtttccgacctgcaggttggaggcagatgtaagtgtaatggacacgcatcacggtgcgtcaaagaccgggatggaaacctagtgtgcgagtgcaagcacaacacagccggaccagagtgtgacagatgcaaaccttttcactatgaccgaccctggcagcgcgcaaccgccagagaagccaacgaatgtgtcgcctgcaattgtaaccttcatgcgaggcgctgtcgtttcaacatggagctttacaaactctctggaaggaaaagtggaggagtctgtctgaactgccgccacaatacagctggtcgccactgccactactgcaaagagggctactatagagacatgtccaagcccatctcccacagaaaggcctgcaaagcctgtgattgccatcctgtgggggccgcgggcaaaacctgtaaccaaaccacaggccaatgcccctgtaaagacggtgtgacgggtatcacatgcaaccgttgtgctaacggctaccagcagagccgatcacccattgccccctgcataaaaattcccatcgctccgcca

SEQ ID NO: 42 - protein, 458 aa, Danio rerio
MVRVSDALVTLVTLCCVLKGTVGGYGMSMFAAQTSPPDPCYDENGHPRRCIPDFVNAAFGKEVRASSTCGKTPSRYCVVTEKGDERHRNCHTCDASDPKKNHPPAYLTDLNNPHNLTCWQSDNYLQYPQNVTLTLSLGKKFEVTYVSLQFCSPRPESMAIFKSMDYGKSWVPFQYYSTQCRKMYNKPSKATITKQNEQEAICTDSHTDMHPLSGGLIAFSTLDGRPSAHDFDNSPVLQDWVTATDIKVTFSRLHTFGDENEDDSELARDSYFYAVSDLQVGGRCKCNGHASRCVKDRDGNLVCECKHNTAGPECDRCKPFHYDRPWQRATAREANECVACNCNLHARRCRFNMELYKLSGRKSGGVCLNCRHNTAGRHCHYCKEGYYRDMSKPISHRKACKACDCHPVGAAGKTCNQTTGQCPCKDGVTGITCNRCANGYQQSRSPIAPCIKIPIAPP

SEQ ID NO: 43 - DNA, 684 bp, Danio rerio
atggtgagagtctctgatgctttggtcactttggtgactctctgctgtgtgctcaaagggactgtcggcggatatggaggagacgaaaacgaggatgactcggagctggccagagattcctatttttacgcagtttccgacctgcaggttggaggcagatgtaagtgtaatggacacgcatcacggtgcgtcaaagaccgggatggaaacctagtgtgcgagtgcaagcacaacacagccggaccagagtgtgacagatgcaaaccttttcactatgaccgaccctggcagcgcgcaaccgccagagaagccaacgaatgtgtcgcctgcaattgtaaccttcatgcgaggcgctgtcgtttcaacatggagctttacaaactctctggaaggaaaagtggaggagtctgtctgaactgccgccacaatacagctggtcgccactgccactactgcaaagagggctactatagagacatgtccaagcccatctcccacagaaaggcctgcaaagcctgtgattgccatcctgtgggggccgcgggcaaaacctgtaaccaaaccacaggccaatgcccctgtaaagacggtgtgacgggtatcacatgcaaccgttgtgctaacggctaccagcagagccgatcacccattgccccctgcataaaaattcccatcgctccgcca

SEQ ID NO: 44 - protein, 228 aa, Danio rerio
MVRVSDALVTLVTLCCVLKGTVGGYGGDENEDDSELARDSYFYAVSDLQVGGRCKCNGHASRCVKDRDGNLVCECKHNTAGPECDRCKPFHYDRPWQRATAREANECVACNCNLHARRCRFNMELYKLSGRKSGGVCLNCRHNTAGRHCHYCKEGYYRDMSKPISHRKACKACDCHPVGAAGKTCNQTTGQCPCKDGVTGITCNRCANGYQQSRSPIAPCIKIPIAPP

SEQ ID NO: 45 - protein, 202 aa, Danio rerio
GDENEDDSELARDSYFYAVSDLQVGGRCKCNGHASRCVKDRDGNLVCECKHNTAGPECDRCKPFHYDRPWQRATAREANECVACNCNLHARRCRFNMELYKLSGRKSGGVCLNCRHNTAGRHCHYCKEGYYRDMSKPISHRKACKACDCHPVGAAGKTCNQTTGQCPCKDGVTGITCNRCANGYQQSRSPIAPCIKIPIAPP

SEQ ID NO: 46 - DNA, 468 bp, Danio rerio
atggtgagagtctctgatgctttggtcactttggtgactctctgctgtgtgctcaaagggactgtcggcggatatggacctgcatcgcctgcctcacccgcttctgtcgcctgcaattgtaaccttcatgcgaggcgctgtcgtttcaacatggagctttacaaactctctggaaggaaaagtggaggagtctgtctgaactgccgccacaatacagctggtcgccactgccactactgcaaagagggctactatagagacatgtccaagcccatctcccacagaaaggcctgcaaagcctgtgattgccatcctgtgggggccgcgggcaaaacctgtaaccaaaccacaggccaatgcccctgtaaagacggtgtgacgggtatcacatgcaaccgttgtgctaacggctaccagcagagccgatcacccattgccccctgcataaaaattcccatcgctccgcca

SEQ ID NO: 47 - protein, 156 aa, Danio rerio
MVRVSDALVTLVTLCCVLKGTVGGYGPASPASPASVACNCNLHARRCRFNMELYKLSGRKSGGVCLNCRHNTAGRHCHYCKEGYYRDMSKPISHRKACKACDCHPVGAAGKTCNQTTGQCPCKDGVTGITCNRCANGYQQSRSPIAPCIKIPIAPP

SEQ ID NO: 48 - protein, 121 aa, Danio rerio
VACNCNLHARRCRFNMELYKLSGRKSGGVCLNCRHNTAGRHCHYCKEGYYRDMSKPISHRKACKACDCHPVGAAGKTCNQTTGQCPCKDGVTGITCNRCANGYQQSRSPIAPCIKIPIAPP

SEQ ID NO: 49 - DNA, 279 bp, Danio rerio
atggtgagagtctctgatgctttggtcactttggtgactctctgctgtgtgctcaaagggactgtcggcggatatggacctgcatcgcctgcctcacccgcttctaaagcctgtgattgccatcctgtgggggccgcgggcaaaacctgtaaccaaaccacaggccaatgcccctgtaaagacggtgtgacgggtatcacatgcaaccgttgtgctaacggctaccagcagagccgatcacccattgccccctgcataaaaattcccatcgctccgcca

SEQ ID NO: 50 - protein, 93 aa, Danio rerio
MVRVSDALVTLVTLCCVLKGTVGGYGPASPASPASKACDCHPVGAAGKTCNQTTGQCPCKDGVTGITCNRCANGYQQSRSPIAPCIKIPIAPP

SEQ ID NO: 51 - protein, 58 aa, Danio rerio
KACDCHPVGAAGKTCNQTTGQCPCKDGVTGITCNRCANGYQQSRSPIAPCIKIPIAPP

SEQ ID NO: 52 - protein, 343 aa, Mus musculus
MAGCPVLRVPTLFLILLLFPELHTAGTLASGSSARNLPETHSHLPSSALWVSQASHHGRRGLGKKDRGPGRPSRAQEGAVVTATKQASQMTLGQPPAGLLQNKELLLGLTLPYPEKEARSPAWERVKKRGREHKRRRDRLRLHRGRAAIRGPSSLMKKVEPSEDRMLEGTMEESSTSLAPTMFFLTMTDGATPTTEESRILPVTSLRPQTQPRSDGEVMPTLDMALFDWTDYEDLKPEVWPSAKKKEKHWSHFTSDGNETSPAEGDPCDHHQDCLPGTCCDLREHLCTPHNRGLNNKCFDDCMCMEGLRCYAKFHRNRRVTRRKGRCVEPETANGDQGSFINI

SEQ ID NO: 53 - protein, 349 aa, Gallus gallus
MAASSTFFSPSLFLCVLVLIDITLAVSLDTDMKLKSENNNHLQNQETWPQQPRSGHHHKHGLAKKGRVLALPVRGQPAGEEALRVGSGAPAMEELVPLGQPAALKQDKDKDVFLGFELPHAERENQSPGSERGKKQNREQRRHSRRDRLKHHRGKTAVGPSSLYKKPESFEQQFQNLQAEEATSPTPTVLPFTALDLVVSTEEPPVLPATSPRSQARLRQDGDVMPTLDMALFDWTDYEDLKPEMWPSAKKKEKRRSKSSNGGNETSSAEGEPCDHHLDCLPGSCCDLREHLCKPHNRGLNNKCYDDCMCTEGLRCYAKFHRNRRVTRRKGRCVEPESANGEQGSFINV

SEQ ID NO: 54 - protein, 21 aa, Felis catus
EVMPTLDMALFDWTDYEDLKP

SEQ ID NO: 55 - protein, 21 aa, Rattus norvegicus
EVMPTLDMALFDWTDYEDLKP

SEQ ID NO: 56 - protein, 21 aa, Mus musculus
EVMPTLDMALFDWTDYEDLKP

SEQ ID NO: 57 - protein, 21 aa, Equus caballus
EVMPTLDMALFDWTDYEDLKP

SEQ ID NO: 58 - protein, 21 aa, Bos taurus
EVMPTLDMALFDWTDYEDLKP

SEQ ID NO: 59 - protein, 21 aa, Sus scrofa
EVMPTLDMALFDWTDYEDLKP

SEQ ID NO: 60 - protein, 21 aa, Canis lupus
EVMPTLDMALFDWTDYEDLRP

SEQ ID NO: 61 - protein, 21 aa, Gallus gallus
DVMPTLDMALFDWTDYEDLKP

SEQ ID NO: 62 - protein, 21 aa, Takifugu rubripes
EVMPTLDMTLFDWTDYEDMKP

SEQ ID NO: 63 - protein, 21 aa, Xenopus tropicalis
DVMPTLDMTLFDWTDYEDMKP

SEQ ID NO: 64 - protein, 48 aa, Danio rerio
CDCHPVGAAGKTCNQTTGQCPCKDGVTGITCNRCANGYQQSRSPIAPC

SEQ ID NO: 65 - protein, 48 aa, Homo sapiens
CDCHPVGAAGKTCNQTTGQCPCKDGVTGITCNRCAKGYQQSRSPIAPC

SEQ ID NO: 66 - DNA, 1029 bp, Mus musculus
atggcagggtgccccgtcctcagggtccccacgctgttcctgatcctcctgctgtttccagagctccacacggcaggcacccttgcatctggatcctctgcccggaacctgccggagacccactcccacctccccagctctgcactgtgggtgtcccaggcaagccatcatggccgtcggggcctggggaagaaagacaggggcccaggaaggcctagccgggcccaggagggggctgtggtcactgctaccaagcaggcttcccagatgacactcggacagccccctgctggccttctgcagaataaggagctgcttctggggctgactttgccctaccccgagaaggaggcccggtctcccgcttgggagagggtgaagaaacgtggcagagaacacaagagacgcagggaccgtctgcgactgcaccgaggccgagctgccatccgtggccccagctccctcatgaagaaggtggaaccctctgaagaccggatgctggagggtaccatggaggagtcttccactagcctggcccccaccatgttcttcctgaccatgacagacggtgccacgcctactacagaagagtcccggatcctgcctgtcacgtccttgcggccccagacacagcccaggtctgacggggaggtgatgcccacactggacatggccttatttgactggacggattatgaagacttaaagccagaggtctggccttctgcaaagaagaaagagaaacactggagtcattttaccagtgatggtaacgagacctcgccagctgagggggatccgtgtgaccatcaccaggattgcttgccaggaacttgctgtgacctccgggaacatctctgcacaccccacaaccgcggcctcaacaacaaatgtttcgacgactgcatgtgcatggaagggctgcgttgctatgccaaattccaccggaaccgcagggtcactcggaggaaggggcgctgcgtggaaccggagacagccaacggggaccagggatctttcatcaacatc

SEQ ID NO: 67 - DNA, 1047 bp, Gallus gallus
atggcagcttcttccaccttcttctctccgtctcttttcctgtgtgtgctggttcttattgacatcacccttgccgtctccctggacactgacatgaagctcaaaagtgagaacaacaaccaccttcaaaaccaagagacgtggcctcagcagcccaggagtgggcaccaccacaagcatggcttggccaagaaagggagggtccttgccctgcctgttagagggcagccagctggggaagaggccctccgagtgggcagtggagctccagccatggaagagctggtgccacttggccagccagcagcgctgaaacaggataaggataaggatgtgttcctgggctttgagctcccacacgctgagcgggagaatcagtcccctgggtctgagaggggaaagaagcagaaccgagagcagcgacggcacagccgcagggacaggctgaaacaccacagagggaagactgccgttgggccaagctccctgtataagaaacctgaaagcttcgagcaacagtttcaaaacctccaggcagaggaagcaaccagcccgacccccaccgtgcttcccttcactgcactggatctggtcgtttccacagaagagcctcctgttcttccagccacgtcgccgcggtcacaggcccgcctcaggcaagatggggatgtgatgcccaccctagatatggcactctttgactggacagattatgaggacctcaaaccagaaatgtggccgtcagctaaaaagaaagagaaacgccgcagtaagagctccaatggtggaaatgaaacctcatcggcagaaggagagccgtgtgaccaccaccttgactgcctcccaggctcttgctgtgacttgcgtgagcacctctgcaaaccacacaatcgaggccttaacaacaaatgctacgatgactgtatgtgcacagaagggctacgctgttatgccaaattccaccggaaccgaagagtgacccgaaggaaagggcgctgtgtggagcctgagtcggccaatggagagcagggatcattcattaatgtt

SEQ ID NO: 68 - DNA, 1338 bp, Artificial Sequence
  fusion protein (zebrafish signal sequence)-(human Netrin1)
atggtggctcctggcttgtgtcaactcttcattctacccgggctcagcatgttcgcgggccaggcggcgcagcccgatccctgctcggacgagaacggccacccgcgccgctgcatcccggactttgtcaatgcggccttcggcaaggacgtgcgcgtgtccagcacctgcggccggcccccggcgcgctactgcgtggtgagcgagcgcggcgaggagcggctgcgctcgtgccacctctgcaacgcgtccgaccccaagaaggcgcacccgcccgccttcctcaccgacctcaacaacccgcacaacctgacgtgctggcagtccgagaactacctgcagttcccgcacaacgtcacgctcacactgtccctcggcaagaagttcgaagtgacctacgtgagcctgcagttctgctcgccgcggcccgagtccatggccatctacaagtccatggactacgggcgcacgtgggtgcccttccagttctactccacgcagtgccgcaagatgtacaaccggccgcaccgcgcgcccatcaccaagcagaacgagcaggaggccgtgtgcaccgactcgcacaccgacatgcgcccgctctcgggcggcctcatcgccttcagcacgctggacgggcggccctcggcgcacgacttcgacaactcgcccgtgctgcaggactgggtcacggccacagacatccgcgtggccttcagccgcctgcacacgttcggcgacgagaacgaggacgactcggagctggcgcgcgactcgtacttctacgcggtgtccgacctgcaggtgggcggccggtgcaagtgcaacggccacgcggcccgctgcgtgcgcgaccgcgacgacagcctggtgtgcgactgcaggcacaacacggccggcccggagtgcgaccgctgcaagcccttccactacgaccggccctggcagcgcgccacagcccgcgaagccaacgagtgcgtggcctgtaactgcaacctgcatgcccggcgctgccgcttcaacatggagctctacaagctttcggggcgcaagagcggaggtgtctgcctcaactgtcgccacaacaccgccggccgccactgccattactgcaaggagggctactaccgcgacatgggcaagcccatcacccaccggaaggcctgcaaagcctgtgattgccaccctgtgggtgctgctggcaaaacctgcaaccaaaccaccggccagtgtccctgcaaggacggcgtgacgggtatcacctgcaaccgctgcgccaaaggctaccagcagagccgctctcccatcgccccctgcataaagatccctgtagcgccgccg

SEQ ID NO: 69 - protein, 446 aa, Artificial Sequence
  fusion protein (zebrafish signal sequence)-(human Netrin1)
MVAPGLCQLFILPGLSMFAGQAAQPDPCSDENGHPRRCIPDFVNAAFGKDVRVSSTCGRPPARYCVVSERGEERLRSCHLCNASDPKKAHPPAFLTDLNNPHNLTCWQSENYLQFPHNVTLTLSLGKKFEVTYVSLQFCSPRPESMAIYKSMDYGRTWVPFQFYSTQCRKMYNRPHRAPITKQNEQEAVCTDSHTDMRPLSGGLIAFSTLDGRPSAHDFDNSPVLQDWVTATDIRVAFSRLHTFGDENEDDSELARDSYFYAVSDLQVGGRCKCNGHAARCVRDRDDSLVCDCRHNTAGPECDRCKPFHYDRPWQRATAREANECVACNCNLHARRCRFNMELYKLSGRKSGGVCLNCRHNTAGRHCHYCKEGYYRDMGKPITHRKACKACDCHPVGAAGKTCNQTTGQCPCKDGVTGITCNRCAKGYQQSRSPIAPCIKIPVAPP

SEQ ID NO: 70 - protein, 26 aa, Danio rerio
MVAPGLCQLFILLLITLSHTLHSSEG

SEQ ID NO: 71 - protein, 23 aa, Danio rerio
MVAPGLCQLFILLLITLSHTLHS

SEQ ID NO: 72 - DNA, 1740 bp, Homo sapiens
atgcctggctggccctgggggctgctgctgacggcaggcacgctcttcgccgccctgagtcctgggccgccggcgcccgccgacccctgccacgatgaggggggtgcgccccgcggctgcgtgccaggactggtgaacgccgccctgggccgcgaggtgctggcttccagcacgtgcgggcggccggccactcgggcctgcgacgcctccgacccgcgacgggcacactcccccgccctccttacttccccagggggcacggccagccctctgtgctggcgctcggagtccctgcctcgggcgcccctcaacgtgactctcacggtgcccctgggcaaggcttttgagctggtcttcgtgagcctgcgcttctgctcagctcccccagcctccgtggccctgctcaagtctcaggaccatggccgcagctgggccccgctgggcttcttctcctcccactgtgacctggactatggccgtctgcctgcccctgccaatggcccagctggcccagggcctgaggccctgtgcttccccgcacccctggcccagcctgatggcagcggccttctggccttcagcatgcaggacagcagccccccaggcctggacctggacagcagcccagtgctccaagactgggtgaccgccaccgacgtccgtgtagtgctcacaaggcctagcacggcaggtgaccccagggacatggaggccgtcgtcccttactcctacgcagccaccgacctccaggtgggcgggcgctgcaagtgcaatggacatgcctcacggtgcctgctggacacacagggccacctgatctgcgactgtcggcatggcaccgagggccctgactgcggccgctgcaagcccttctactgcgacaggccatggcagcgggccactgcccgggaatcccacgcctgcctcgcttgctcctgcaacggccatgcccgccgctgccgcttcaacatggagctgtaccgactgtccggccgccgcagcgggggtgtctgtctcaactgccggcacaacaccgccggccgccactgccactactgccgggagggcttctatcgagaccctggccgtgccctgagtgaccgtcgggcttgcagggcctgcgactgtcacccggttggtgctgctggcaagacctgcaaccagaccacaggccagtgtccctgcaaggatggcgtcactggcctcacctgcaaccgctgcgcgcctggcttccagcaaagccgctccccagtggcgccctgtgttaagacccctatccctggacccactgaggacagcagccctgtgcagccccaggactgtgactcgcactgcaaacctgcccgtggcagctaccgcatcagcctaaagaagttctgcaagaaggactatgcggtgcaggtggcggtgggtgcgcgcggcgaggcgcgcggcgcgtggacacgcttcccggtggcggtgctcgccgtgttccggagcggagaggagcgcgcgcggcgcgggagtagcgcgctgtgggtgcccgccggggatgcggcctgcggctgcccgcgcctgctccccggccgccgctacctcctgctggggggcgggcctggagccgcggctgggggcgcggggggccgggggcccgggctcatcgccgcccgcggaagcctcgtgctaccctggagggacgcgtggacgcggcgcctgcggaggctgcagcgacgcgaacggcgggggcgctgcagcgccgcc

SEQ ID NO: 73 - protein, 577 aa, Homo sapiens
MSMFAAQTSPPDPCYDENGHPRRCIPDFVNAAFGKEVRASSTCGKTPSRYCVVTEKGDERHRNCHTCDASDPKKNHPPAYLTDLNNPHNLTCWQSDNYLQYPQNVTLTLSLGKKFEVTYVSLQFCSPRPESMAIFKSMDYGKSWVPFQYYSTQCRKMYNKPSKATITKQNEQEAICTDSHTDMHPLSGGLIAFSTLDGRPSAHDFDNSPVLQDWVTATDIKVTFSRLHTFGDENEDDSELARDSYFYAVSDLQVGGRCKCNGHASRCVKDRDGNLVCECKHNTAGPECDRCKPFHYDRPWQRATAREANECVACNCNLHARRCRFNMELYKLSGRKSGGVCLNCRHNTAGRHCHYCKEGYYRDMSKPISHRKACKACDCHPVGAAGKTCNQTTGQCPCKDGVTGITCNRCANGYQQSRSPIAPCIKIPIAPPTTTASSTEEPSDCESYCKASKGKLKINMKKYCKKDYAVQVHILKADKAGEWWKFTVNIISVYKQGESRIRRGDQFLWVRAKDVACKCPKIKSGKKYLLLGNDEDSPGQSGMVADKGSLVIQWRDTWARRLRKFQQREKKGKCKKA

SEQ ID NO: 74 - DNA, 501 bp, Homo sapiens
tgcaagtgcaatggacatgcctcacggtgcctgctggacacacagggccacctgatctgcgactgtcggcatggcaccgagggccctgactgcggccgctgcaagcccttctactgcgacaggccatggcagcgggccactgcccgggaatcccacgcctgcctcgcttgctcctgcaacggccatgcccgccgctgccgcttcaacatggagctgtaccgactgtccggccgccgcagcgggggtgtctgtctcaactgccggcacaacaccgccggccgccactgccactactgccgggagggcttctatcgagaccctggccgtgccctgagtgaccgtcgggcttgcagggcctgcgactgtcacccggttggtgctgctggcaagacctgcaaccagaccacaggccagtgtccctgcaaggatggcgtcactggcctcacctgcaaccgctgcgcgcctggcttccagcaaagccgctccccagtggcgccctgt

SEQ ID NO: 75 - protein, 167 aa, Homo sapiens
CKCNGHASRCLLDTQGHLICDCRHGTEGPDCGRCKPFYCDRPWQRATARESHACLACSCNGHARRCRFNMELYRLSGRRSGGVCLNCRHNTAGRHCHYCREGFYRDPGRALSDRRACRACDCHPVGAAGKTCNQTTGQCPCKDGVTGLTCNRCAPGFQQSRSPVAPC

SEQ ID NO: 76 - DNA, 144 bp, Homo sapiens
tgcgactgtcacccggttggtgctgctggcaagacctgcaaccagaccacaggccagtgtccctgcaaggatggcgtcactggcctcacctgcaaccgctgcgcgcctggcttccagcaaagccgctccccagtggcgccctgt

SEQ ID NO: 77 - protein, 48 aa, Homo sapiens
CDCHPVGAAGKTCNQTTGQCPCKDGVTGLTCNRCAPGFQQSRSPVAPC

SEQ ID NO: 78 - protein, 52 aa, Homo sapiens
CSCHPVGSAVLPANSVTFCDPSNGDCPCKPGVAGRRCDRCMVGYWGFGDYGC

SEQ ID NO: 79 - protein, 48 aa, Danio rerio; identical to SEQ ID NO: 65

SEQ ID NO: 80 - DNA, 25 bp, Artificial Sequence
  ntn1a morpholino
atgatggacttaccgacacattcgt

SEQ ID NO: 81 - DNA, 25 bp, Artificial Sequence
  ntn1b morpholino
cgcacgttaccaaaatccttatcat